European Patent Application EP 4 599 835 A1, published August 13, 2025. Title: ウイルス感染抑制剤. Applicant: 日環科学株式会社. The sequence listing filed with the application follows.

SEQUENCE LISTING (3 sequences)

SEQ ID NO: 1 - DNA, 630 bp, Caldibacillus
  source 1..630: mol_type = genomic DNA
ttatttcattaaggaaacaccttggaaaatttttgcccaatatggatcattttcatcccaaatttctttatttggcagttcaacaagagttactgaggaaagcggatacggtttttcaatcatatgacttatgtttttatggtggactaatagaatgtgaaaatctccggctaccatattggacaaaatcgtctccaattcttttacatcttcaaattttgcttcatttgcttcagttcggatgaataaaattcgtttactcgtattcattttttcaagaaaccgattaattcttctgtcatattttgcttttacttccgcatacccgcctaaatgagttaatgtgtttttatcggttttaaaatcatggttaaagccaatatcataaacaaagtcatgaacatataaatctgtaggcgagagatagcgatcgggttttaaatgattgatattcaaaaaatcggaaaaacggtttttaatcagcaaattgacttttgataattgtggggaaccaacccaatccagcacacccgaaaacggacgtaactgaaacttccgcaattgcatggcagctaaacaaagatgccctaaactgaaaatggaatcatacgtaccctttaatttatgcaa

SEQ ID NO: 2 - DNA, 324 bp, Caldibacillus
  source 1..324: mol_type = genomic DNA
tcacctcaggataagcggcaaggtcggcgaccgtattttgcccgcttcgaaatcgtggctggaaatgatggaattggcgtcatccgtcacccagatcattccggtttccgttaccccgcctacccgtaaattttccagctccataaatcctttgaacctggtgtcgatcagccggcagacatcgtcaagattcggcgaagccacccagtcgaatacgccggcgtagggacggagattgtttttctcgagctgcagcgaagacaaacataggtctcccaagctgaaaatcgcatcgtagccgccttttaaatctgccagtttcat

SEQ ID NO: 3 - DNA, 172 bp, Caldibacillus
  source 1..172: mol_type = genomic DNA
gatggctaagtttgatgatttcgatttggacatcgttgtcaaaaaacaagataccactgtacaaccgaatgttacaagtaaatctctttgtacgcctggttgtatcacaggtattttaatgtgcttaactcaaaactcctgtgtatcttgtaactcttgcatcaaatgttaa